European Patent Specification EP 3 364 967 B1, published May 20, 2026. Title: Novel ferroportin inhibitors. Applicant: Vifor (International) AG. The sequence listing filed with the application follows.

SEQUENCE LISTING (3 sequences)

SEQ ID NO: 1 - protein, 9 aa, human
DTHFPICIF

SEQ ID NO: 2 - DNA, 21 bp, artificial
  forward primer
caggtttgtgagcatcctgaa

SEQ ID NO: 3 - DNA, 19 bp, artificial
  reverse primer
ggcggcgactaaggagagg